European Patent Application EP 4 368 637 A2, published May 15, 2024. Title: METHODS FOR BREAKING IMMUNOLOGICAL TOLERANCE USING MULTIPLE GUIDE RNAS. Applicant: Regeneron Pharmaceuticals, Inc. The sequence listing filed with the application follows.

SEQUENCE LISTING (152 sequences)

SEQ ID NO: 1-3 - skipped (3 entries)

SEQ ID NO: 4 - DNA, 20 bp, synthetic construct
  misc_feature 1..20: note = C5 (Hc) gRNA A DNA-targeting segment (100 bp from target locus endpoint)
  source 1..20: mol_type = other DNA
atcacaaaccagttaaccgg

SEQ ID NO: 5 - DNA, 20 bp, synthetic construct
  misc_feature 1..20: note = C5 (Hc) gRNA B DNA-targeting segment (500 bp from target locus endpoint)
  source 1..20: mol_type = other DNA
tttcagacgagccgacccgg

SEQ ID NO: 6 - DNA, 20 bp, synthetic construct
  misc_feature 1..20: note = C5 (Hc) gRNA C DNA-targeting segment (38200 and 37500 bp from target locus endpoints)
  source 1..20: mol_type = other DNA
tgtgtgtcatagcgatgtcg

SEQ ID NO: 7 - DNA, 20 bp, synthetic construct
  misc_feature 1..20: note = C5 (Hc) gRNA D DNA-targeting segment (43500 and 32200 bp from target locus endpoints)
  source 1..20: mol_type = other DNA
aacaggtaccctatcctcac

SEQ ID NO: 8 - DNA, 20 bp, synthetic construct
  misc_feature 1..20: note = C5 (Hc) gRNA E DNA-targeting segment (500 bp from target locus endpoint)
  source 1..20: mol_type = other DNA
ggcccggacctagtctctct

SEQ ID NO: 9 - DNA, 20 bp, synthetic construct
  misc_feature 1..20: note = C5 (Hc) gRNA E2 DNA-targeting segment (100 bp from target locus endpoint)
  source 1..20: mol_type = other DNA
tcgtggttgcatgcgcactg

SEQ ID NO: 10 - DNA, 20 bp, synthetic construct
  misc_feature 1..20: note = Lrp5 gRNA A DNA-targeting segment (50 bp from target locus end point)
  source 1..20: mol_type = other DNA
gggaacccacagcatactcc

SEQ ID NO: 11 - DNA, 20 bp, synthetic construct
  misc_feature 1..20: note = Lrp5 gRNA B DNA-targeting segment (500 bp from target locus end point)
  source 1..20: mol_type = other DNA
gaatcatgcacggctacccc

SEQ ID NO: 12 - DNA, 20 bp, synthetic construct
  misc_feature 1..20: note = Lrp5 gRNA B2 DNA-targeting segment (1000 bp from target locus end point)
  source 1..20: mol_type = other DNA
tgctcctatggggaggcgcg

SEQ ID NO: 13 - DNA, 20 bp, synthetic construct
  misc_feature 1..20: note = Lrp5 gRNA C DNA-targeting segment (29900 and 38430 bp from target locus end points)
  source 1..20: mol_type = other DNA
actgagatcaatgaccccga

SEQ ID NO: 14 - DNA, 20 bp, synthetic construct
  misc_feature 1..20: note = Lrp5 gRNA D DNA-targeting segment (29950 and 38380 bp from target locus end points)
  source 1..20: mol_type = other DNA
gggtcgcccggaacctctac

SEQ ID NO: 15 - DNA, 20 bp, synthetic construct
  misc_feature 1..20: note = Lrp5 gRNA E2 DNA-targeting segment (1000 bp from target locus end point)
  source 1..20: mol_type = other DNA
cttggataacattgataccc

SEQ ID NO: 16 - DNA, 20 bp, synthetic construct
  misc_feature 1..20: note = Lrp5 gRNA E DNA-targeting segment (500 bp from target locus end point)
  source 1..20: mol_type = other DNA
ggggcagagcccttatatca

SEQ ID NO: 17 - DNA, 20 bp, synthetic construct
  misc_feature 1..20: note = Lrp5 gRNA F DNA-targeting segment (50 bp from target locus end point)
  source 1..20: mol_type = other DNA
tcgctcacattaatccctag

SEQ ID NO: 18 - DNA, 20 bp, synthetic construct
  misc_feature 1..20: note = Ror1 gRNA A DNA-targeting segment (200 bp from target locus end point)
  source 1..20: mol_type = other DNA
tgtgggcctttgctgatcac

SEQ ID NO: 19 - DNA, 20 bp, synthetic construct
  misc_feature 1..20: note = Ror1 gRNA B DNA-targeting segment (1000 bp from target locus end point)
  source 1..20: mol_type = other DNA
aatctatgatcctatggcct

SEQ ID NO: 20 - DNA, 20 bp, synthetic construct
  misc_feature 1..20: note = Ror1 gRNA D DNA-targeting segment (54300 and 55500 bp from target locus end points)
  source 1..20: mol_type = other DNA
tgccaatagcagtgacttga

SEQ ID NO: 21 - DNA, 20 bp, synthetic construct
  misc_feature 1..20: note = Ror1 gRNA C DNA-targeting segment (54500 and 55300 bp from target locus end points)
  source 1..20: mol_type = other DNA
gggaagaatgggctattgtc

SEQ ID NO: 22 - DNA, 20 bp, synthetic construct
  misc_feature 1..20: note = Ror1 gRNA E DNA-targeting segment (1000 bp from target locus end point)
  source 1..20: mol_type = other DNA
ggttgtttgtgctgatgacg

SEQ ID NO: 23 - DNA, 20 bp, synthetic construct
  misc_feature 1..20: note = Ror1 gRNA F DNA-targeting segment (200 bp from target locus end point)
  source 1..20: mol_type = other DNA
ccgtcctaggccttctacgt

SEQ ID NO: 24 - DNA, 20 bp, synthetic construct
  misc_feature 1..20: note = Trpa1 gRNA A DNA-targeting segment (100 bp from target locus end point)
  source 1..20: mol_type = other DNA
gtactggggaatcggtggtc

SEQ ID NO: 25 - DNA, 20 bp, synthetic construct
  misc_feature 1..20: note = Trpa1 gRNA A2 DNA-targeting segment (500 bp from target locus end point)
  source 1..20: mol_type = other DNA
cacgcactccaaatttatcc

SEQ ID NO: 26 - DNA, 20 bp, synthetic construct
  misc_feature 1..20: note = Trpa1 gRNA B DNA-targeting segment (1000 bp from target locus end point)
  source 1..20: mol_type = other DNA
ctaagtgtgtatcagtacat

SEQ ID NO: 27 - DNA, 20 bp, synthetic construct
  misc_feature 1..20: note = Trpa1 gRNA C DNA-targeting segment (25600 and 19740 bp from target locus end points)
  source 1..20: mol_type = other DNA
tgccctgcacaataagcgca

SEQ ID NO: 28 - DNA, 20 bp, synthetic construct
  misc_feature 1..20: note = Trpa1 gRNA D DNA-targeting segment (26970 and 18370 bp from target locus end points)
  source 1..20: mol_type = other DNA
actcattgaaacgttatggc

SEQ ID NO: 29 - DNA, 20 bp, synthetic construct
  misc_feature 1..20: note = Trpa1 gRNA E2 DNA-targeting segment (1000 bp from target locus end point)
  source 1..20: mol_type = other DNA
agtaagggtggattaaattc

SEQ ID NO: 30 - DNA, 20 bp, synthetic construct
  misc_feature 1..20: note = Trpa1 gRNA E DNA-targeting segment (500 bp from target locus end point)
  source 1..20: mol_type = other DNA
gccatctagattcatgtaac

SEQ ID NO: 31 - DNA, 20 bp, synthetic construct
  misc_feature 1..20: note = Trpa1 gRNA F DNA-targeting segment (100 bp from target locus end point)
  source 1..20: mol_type = other DNA
gactagaaatgttctgcacc

SEQ ID NO: 32 - DNA, 21 bp, synthetic construct
  misc_feature 1..21: note = 190045 forward primer
  source 1..21: mol_type = other DNA
gagctcatagccaacagcttg

SEQ ID NO: 33 - DNA, 20 bp, synthetic construct
  misc_feature 1..20: note = 190061 forward primer
  source 1..20: mol_type = other DNA
atgcatcagatcacgctcag

SEQ ID NO: 34 - DNA, 20 bp, synthetic construct
  misc_feature 1..20: note = 190068 forward primer
  source 1..20: mol_type = other DNA
gtccttgtggcatttccaac

SEQ ID NO: 35 - DNA, 24 bp, synthetic construct
  misc_feature 1..24: note = 190030 forward primer
  source 1..24: mol_type = other DNA
ccagtatggtgtcagttaatagcg

SEQ ID NO: 36 - DNA, 19 bp, synthetic construct
  misc_feature 1..19: note = 190033 forward primer (same as forward primer for SV 48.3 in Fig. 6)
  source 1..19: mol_type = other DNA
ctgtgcagaaagcagcctc

SEQ ID NO: 37 - DNA, 20 bp, synthetic construct
  misc_feature 1..20: note = 190013 forward primer
  source 1..20: mol_type = other DNA
cctctccctctaggcacctg

SEQ ID NO: 38 - DNA, 20 bp, synthetic construct
  misc_feature 1..20: note = 190045 reverse primer
  source 1..20: mol_type = other DNA
tctttaagggctccgttgtc

SEQ ID NO: 39 - DNA, 20 bp, synthetic construct
  misc_feature 1..20: note = 190061 reverse primer
  source 1..20: mol_type = other DNA
aagaccaaccattcacccag

SEQ ID NO: 40 - DNA, 20 bp, synthetic construct
  misc_feature 1..20: note = 190068 reverse primer
  source 1..20: mol_type = other DNA
ttcccagtccaagtcaaagg

SEQ ID NO: 41 - DNA, 20 bp, synthetic construct
  misc_feature 1..20: note = 190030 reverse primer
  source 1..20: mol_type = other DNA
ctgttatctgcaaggcaccc

SEQ ID NO: 42 - DNA, 20 bp, synthetic construct
  misc_feature 1..20: note = 190033 reverse primer (same as reverse primer for SV 48.3 in Fig. 6)
  source 1..20: mol_type = other DNA
acaactggatcctgattcgc

SEQ ID NO: 43 - DNA, 20 bp, synthetic construct
  misc_feature 1..20: note = 190013 reverse primer
  source 1..20: mol_type = other DNA
taagagggcatgggtgagac

SEQ ID NO: 44 - DNA, 20 bp, synthetic construct
  misc_feature 1..20: note = C2 probe (B6) - SNV 0.32 in Fig. 6
  source 1..20: mol_type = other DNA
aattcagaagacctatcgta

SEQ ID NO: 45 - DNA, 21 bp, synthetic construct
  misc_feature 1..21: note = T3 probe (B6) - SNV 1.2 in Fig. 6
  source 1..21: mol_type = other DNA
tatgtgtataggtgtttggat

SEQ ID NO: 46 - DNA, 19 bp, synthetic construct
  misc_feature 1..19: note = T6 probe (B6) - SNV 11.1 in Fig. 6
  source 1..19: mol_type = other DNA
tacattgctaaatgaaacc

SEQ ID NO: 47 - DNA, 16 bp, synthetic construct
  misc_feature 1..16: note = T7 probe (B6) - SNV 13.2 in Fig. 6
  source 1..16: mol_type = other DNA
cgcagtcatgcacata

SEQ ID NO: 48 - DNA, 20 bp, synthetic construct
  misc_feature 1..20: note = T8 probe (B6) - SNV 17.5 in Fig. 6
  source 1..20: mol_type = other DNA
ttataaagcccagtatgtac

SEQ ID NO: 49 - DNA, 14 bp, synthetic construct
  misc_feature 1..14: note = T9 probe (B6) - SNV 25.8 in Fig. 6
  source 1..14: mol_type = other DNA
tgctgcataatcag

SEQ ID NO: 50 - DNA, 18 bp, synthetic construct
  misc_feature 1..18: note = T10 probe (B6) - SNV 33.0 in Fig. 6
  source 1..18: mol_type = other DNA
tcaggagtgaattggata

SEQ ID NO: 51 - DNA, 16 bp, synthetic construct
  misc_feature 1..16: note = T11 probe (B6) - SNV 38.3 in Fig. 6
  source 1..16: mol_type = other DNA
ctgctacttacctttg

SEQ ID NO: 52 - DNA, 13 bp, synthetic construct
  misc_feature 1..13: note = T13 probe (B6) - SNV 49.6 in Fig. 6
  source 1..13: mol_type = other DNA
aggaggaaaacgc

SEQ ID NO: 53 - DNA, 17 bp, synthetic construct
  misc_feature 1..17: note = T14 probe (B6) - SNV 57.2 in Fig. 6
  source 1..17: mol_type = other DNA
cctttgttcctcataag

SEQ ID NO: 54 - DNA, 20 bp, synthetic construct
  misc_feature 1..20: note = C2 probe (129) - SNV 0.32 in Fig. 6
  source 1..20: mol_type = other DNA
aattcagaagacctattgta

SEQ ID NO: 55 - DNA, 21 bp, synthetic construct
  misc_feature 1..21: note = T3 probe (129) - SNV 1.2 in Fig. 6
  source 1..21: mol_type = other DNA
tatgtgtataggtgtttgcat

SEQ ID NO: 56 - DNA, 16 bp, synthetic construct
  misc_feature 1..16: note = T6 probe (129) - SNV 11.1 in Fig. 6
  source 1..16: mol_type = other DNA
cattgctacatgaaac

SEQ ID NO: 57 - DNA, 16 bp, synthetic construct
  misc_feature 1..16: note = T7 probe (129) - SNV 13.2 in Fig. 6
  source 1..16: mol_type = other DNA
cgcagtcatgcacgta

SEQ ID NO: 58 - DNA, 23 bp, synthetic construct
  misc_feature 1..23: note = T8 probe (129) - SNV 17.5 in Fig. 6
  source 1..23: mol_type = other DNA
tgagaatttataaagcccaatat

SEQ ID NO: 59 - DNA, 14 bp, synthetic construct
  misc_feature 1..14: note = T9 probe (129) - SNV 25.8 in Fig. 6
  source 1..14: mol_type = other DNA
tgctgcatgatcag

SEQ ID NO: 60 - DNA, 15 bp, synthetic construct
  misc_feature 1..15: note = T10 probe (129) - SNV 33.0 in Fig. 6
  source 1..15: mol_type = other DNA
tcaggagtgaatcgg

SEQ ID NO: 61 - DNA, 16 bp, synthetic construct
  misc_feature 1..16: note = T11 probe (129) - SNV 38.3 in Fig. 6
  source 1..16: mol_type = other DNA
ctgctagttacctttg

SEQ ID NO: 62 - DNA, 15 bp, synthetic construct
  misc_feature 1..15: note = T13 probe (129) - SNV 49.6 in Fig. 6
  source 1..15: mol_type = other DNA
aggaggaagacgcag

SEQ ID NO: 63 - DNA, 17 bp, synthetic construct
  misc_feature 1..17: note = T14 probe (129) - SNV 57.2 in Fig. 6
  source 1..17: mol_type = other DNA
ctttgttcttcataagc

SEQ ID NO: 64 - DNA, 25 bp, synthetic construct
  misc_feature 1..25: note = C2 forward primer - SNV 0.32 in Fig. 6
  source 1..25: mol_type = other DNA
atgagggatttccttaatcagacaa

SEQ ID NO: 65 - DNA, 29 bp, synthetic construct
  misc_feature 1..29: note = T3 forward primer - SNV 1.2 in Fig. 6
  source 1..29: mol_type = other DNA
tggtatgtttattcttactcaaggttttg

SEQ ID NO: 66 - DNA, 22 bp, synthetic construct
  misc_feature 1..22: note = T6 forward primer - SNV 11.1 in Fig. 6
  source 1..22: mol_type = other DNA
gggcaactgatggaaagaactc

SEQ ID NO: 67 - DNA, 23 bp, synthetic construct
  misc_feature 1..23: note = T7 forward primer - SNV 13.2 in Fig. 6
  source 1..23: mol_type = other DNA
gactgacgcacaaacttgtcctt

SEQ ID NO: 68 - DNA, 26 bp, synthetic construct
  misc_feature 1..26: note = T8 forward primer - SNV 17.5 in Fig. 6
  source 1..26: mol_type = other DNA
cccaaagcatataacaagaacaaatg

SEQ ID NO: 69 - DNA, 18 bp, synthetic construct
  misc_feature 1..18: note = T9 forward primer - SNV 25.8 in Fig. 6
  source 1..18: mol_type = other DNA
gcaggacgcaggcgttta

SEQ ID NO: 70 - DNA, 23 bp, synthetic construct
  misc_feature 1..23: note = T10 forward primer - SNV 33.0 in Fig. 6
  source 1..23: mol_type = other DNA
gcatcctcatggcagtctacatc

SEQ ID NO: 71 - DNA, 20 bp, synthetic construct
  misc_feature 1..20: note = T11 forward primer - SNV 38.3 in Fig. 6
  source 1..20: mol_type = other DNA
cctgccccttgatgagtgtt

SEQ ID NO: 72 - DNA, 23 bp, synthetic construct
  misc_feature 1..23: note = T13 forward primer - SNV 49.6 in Fig. 6
  source 1..23: mol_type = other DNA
ccctctttgatatgctcgtgtgt

SEQ ID NO: 73 - DNA, 22 bp, synthetic construct
  misc_feature 1..22: note = T14 forward primer - SNV 57.2 in Fig. 6
  source 1..22: mol_type = other DNA
tcccacaggtccatgtctttaa

SEQ ID NO: 74 - DNA, 28 bp, synthetic construct
  misc_feature 1..28: note = C2 reverse primer - SNV 0.32 in Fig. 6
  source 1..28: mol_type = other DNA
agactacaatgagctaccatcataaggt

SEQ ID NO: 75 - DNA, 24 bp, synthetic construct
  misc_feature 1..24: note = T3 reverse primer - SNV 1.2 in Fig. 6
  source 1..24: mol_type = other DNA
caaccatctaaaactccagttcca

SEQ ID NO: 76 - DNA, 28 bp, synthetic construct
  misc_feature 1..28: note = T6 reverse primer - SNV 11.1 in Fig. 6
  source 1..28: mol_type = other DNA
tgtgtaacaggacagttgaatgtagaga

SEQ ID NO: 77 - DNA, 19 bp, synthetic construct
  misc_feature 1..19: note = T7 reverse primer - SNV 13.2 in Fig. 6
  source 1..19: mol_type = other DNA
cttaaaacccgccctgcat

SEQ ID NO: 78 - DNA, 26 bp, synthetic construct
  misc_feature 1..26: note = T8 reverse primer - SNV 17.5 in Fig. 6
  source 1..26: mol_type = other DNA
ctacaggagatgtggctgttctatgt

SEQ ID NO: 79 - DNA, 22 bp, synthetic construct
  misc_feature 1..22: note = T9 reverse primer - SNV 25.8 in Fig. 6
  source 1..22: mol_type = other DNA
tcagcgtgattcgcttgtagtc

SEQ ID NO: 80 - DNA, 26 bp, synthetic construct
  misc_feature 1..26: note = T10 reverse primer - SNV 33.0 in Fig. 6
  source 1..26: mol_type = other DNA
tgcatagctgtttgaataatgacaag

SEQ ID NO: 81 - DNA, 21 bp, synthetic construct
  misc_feature 1..21: note = T11 reverse primer - SNV 38.3 in Fig. 6
  source 1..21: mol_type = other DNA
tgcagcatctctgtcaagcaa

SEQ ID NO: 82 - DNA, 24 bp, synthetic construct
  misc_feature 1..24: note = T13 reverse primer - SNV 49.6 in Fig. 6
  source 1..24: mol_type = other DNA
gcaacaacataacccacagcataa

SEQ ID NO: 83 - DNA, 23 bp, synthetic construct
  misc_feature 1..23: note = T14 reverse primer - SNV 57.2 in Fig. 6
  source 1..23: mol_type = other DNA
gctaagcgtttggaagaaattcc

SEQ ID NO: 84 - DNA, 20 bp, synthetic construct
  misc_feature 1..20: note = Forward primer for SV 13.7 in Fig. 6
  source 1..20: mol_type = other DNA
taggctctaaggatgctggc

SEQ ID NO: 85 - DNA, 20 bp, synthetic construct
  misc_feature 1..20: note = Reverse primer for SV 13.7 in Fig. 6
  source 1..20: mol_type = other DNA
aagcagcttcaaaccctctg

SEQ ID NO: 86 - DNA, 20 bp, synthetic construct
  misc_feature 1..20: note = Forward primer for SV 20.0 in Fig. 6
  source 1..20: mol_type = other DNA
ttacttggccttggaactgc

SEQ ID NO: 87 - DNA, 21 bp, synthetic construct
  misc_feature 1..21: note = Reverse primer for SV 20.0 in Fig. 6
  source 1..21: mol_type = other DNA
tgattcgtaatcgtcactgcc

SEQ ID NO: 88 - DNA, 20 bp, synthetic construct
  misc_feature 1..20: note = Forward primer for SV 36.9 in Fig. 6
  source 1..20: mol_type = other DNA
tcctgtcccgagaaactgtc

SEQ ID NO: 89 - DNA, 20 bp, synthetic construct
  misc_feature 1..20: note = Reverse primer for SV 36.9 in Fig. 6
  source 1..20: mol_type = other DNA
agctggctttcagagagctg

SEQ ID NO: 90 - DNA, 20 bp, synthetic construct
  misc_feature 1..20: note = Forward primer for SV 56.7 in Fig. 6
  source 1..20: mol_type = other DNA
ttagaaagtgccaaccaggc

SEQ ID NO: 91 - DNA, 20 bp, synthetic construct
  misc_feature 1..20: note = Reverse primer for SV 56.7 in Fig. 6
  source 1..20: mol_type = other DNA
ctctggctaggaacaatggc

SEQ ID NO: 92 - DNA, 25 bp, synthetic construct
  misc_feature 1..25: note = m-lr-f primer for Lrp5 locus
  source 1..25: mol_type = other DNA
gttaggtgcagggtctactcagctg

SEQ ID NO: 93 - DNA, 20 bp, synthetic construct
  misc_feature 1..20: note = m-5'-f primer for Lrp5 locus
  source 1..20: mol_type = other DNA
ggaggagaggagaagcagcc

SEQ ID NO: 94 - DNA, 20 bp, synthetic construct
  misc_feature 1..20: note = m-A primer for Lrp5 locus
  source 1..20: mol_type = other DNA
ggaggagaggagaagcagcc

SEQ ID NO: 95 - DNA, 26 bp, synthetic construct
  misc_feature 1..26: note = h-lr-r primer for Lrp5 locus
  source 1..26: mol_type = other DNA
gcaaacagccttcttcccacattcgg

SEQ ID NO: 96 - DNA, 24 bp, synthetic construct
  misc_feature 1..24: note = m-5'-r primer for Lrp5 locus
  source 1..24: mol_type = other DNA
ttgctttcagtagttcaggtgtgc

SEQ ID NO: 97 - DNA, 20 bp, synthetic construct
  misc_feature 1..20: note = h-5'-r primer for Lrp5 locus
  source 1..20: mol_type = other DNA
ggcgttgtcaggaagttgcc

SEQ ID NO: 98 - DNA, 22 bp, synthetic construct
  misc_feature 1..22: note = m-F primer for Lrp5 locus
  source 1..22: mol_type = other DNA
tgaagttgagaggcacatgagg

SEQ ID NO: 99 - DNA, 24 bp, synthetic construct
  misc_feature 1..24: note = m-E2 primer for Lrp5 locus
  source 1..24: mol_type = other DNA
tagagtagccacaggcagcaaagc

SEQ ID NO: 100 - DNA, 22 bp, synthetic construct
  misc_feature 1..22: note = 7064retU forward primer
  source 1..22: mol_type = other DNA
cctcctgagctttcctttgcag

SEQ ID NO: 101 - DNA, 25 bp, synthetic construct
  misc_feature 1..25: note = 7064retU reverse primer
  source 1..25: mol_type = other DNA
cctagacaacacagacactgtatca

SEQ ID NO: 102 - DNA, 23 bp, synthetic construct
  misc_feature 1..23: note = 7064retU TAQMAN probe
  source 1..23: mol_type = other DNA
ttctgcccttgaaaaggagaggc

SEQ ID NO: 103 - DNA, 18 bp, synthetic construct
  misc_feature 1..18: note = 7064retD forward primer
  source 1..18: mol_type = other DNA
cctctgaggccacctgaa

SEQ ID NO: 104 - DNA, 23 bp, synthetic construct
  misc_feature 1..23: note = 7064retD reverse primer
  source 1..23: mol_type = other DNA
ccctgacaagttctgccttctac

SEQ ID NO: 105 - DNA, 21 bp, synthetic construct
  misc_feature 1..21: note = 7064retD TAQMAN probe
  source 1..21: mol_type = other DNA
tgcccaagcctctgcagcttt

SEQ ID NO: 106 - DNA, 19 bp, synthetic construct
  misc_feature 1..19: note = 7140retU forward primer
  source 1..19: mol_type = other DNA
cccagcatctgacgacacc

SEQ ID NO: 107 - DNA, 21 bp, synthetic construct
  misc_feature 1..21: note = 7140retU reverse primer
  source 1..21: mol_type = other DNA
gaccactgtgggcatctgtag

SEQ ID NO: 108 - DNA, 27 bp, synthetic construct
  misc_feature 1..27: note = 7140retU TAQMAN probe
  source 1..27: mol_type = other DNA
ccgagtctgctgttactgttagcatca

SEQ ID NO: 109 - DNA, 20 bp, synthetic construct
  misc_feature 1..20: note = 7140retD forward primer
  source 1..20: mol_type = other DNA
cccgacaccttctgagcatg

SEQ ID NO: 110 - DNA, 21 bp, synthetic construct
  misc_feature 1..21: note = 7140retD reverse primer
  source 1..21: mol_type = other DNA
tgcaggctgagtcaggatttg

SEQ ID NO: 111 - DNA, 25 bp, synthetic construct
  misc_feature 1..25: note = 7140retD TAQMAN probe
  source 1..25: mol_type = other DNA
tagtcacgttttgtgacaccccaga

SEQ ID NO: 112 - DNA, 20 bp, synthetic construct
  misc_feature 1..20: note = Folh1 gRNA A DNA-targeting segment
  source 1..20: mol_type = other DNA
tgaaccaattgtgtagcctt

SEQ ID NO: 113 - DNA, 20 bp, synthetic construct
  misc_feature 1..20: note = Folh1 gRNA A2 DNA-targeting segment
  source 1..20: mol_type = other DNA
aatagtggtaaagcaccatg

SEQ ID NO: 114 - DNA, 20 bp, synthetic construct
  misc_feature 1..20: note = Folh1 gRNA B DNA-targeting segment
  source 1..20: mol_type = other DNA
gtgtgctaaggatcgaagtc

SEQ ID NO: 115 - DNA, 20 bp, synthetic construct
  misc_feature 1..20: note = Folh1 gRNA C DNA-targeting segment
  source 1..20: mol_type = other DNA
caccgagatgcttgggtatt

SEQ ID NO: 116 - DNA, 20 bp, synthetic construct
  misc_feature 1..20: note = Folh1 gRNA D DNA-targeting segment
  source 1..20: mol_type = other DNA
tgtaaccgccctgaatgacc

SEQ ID NO: 117 - DNA, 20 bp, synthetic construct
  misc_feature 1..20: note = Folh1 gRNA E DNA-targeting segment
  source 1..20: mol_type = other DNA
aaaagggcatcataaatccc

SEQ ID NO: 118 - DNA, 20 bp, synthetic construct
  misc_feature 1..20: note = Folh1 gRNA E2 DNA-targeting segment
  source 1..20: mol_type = other DNA
tcaaaaatagtcatacacct

SEQ ID NO: 119 - DNA, 20 bp, synthetic construct
  misc_feature 1..20: note = Folh1 gRNA F DNA-targeting segment
  source 1..20: mol_type = other DNA
ggtctctagtacattgtaga

SEQ ID NO: 120 - DNA, 20 bp, synthetic construct
  misc_feature 1..20: note = Adamts5 gRNA A DNA-targeting segment
  source 1..20: mol_type = other DNA
ggtggtggtgctgacggaca

SEQ ID NO: 121 - DNA, 20 bp, synthetic construct
  misc_feature 1..20: note = Adamts5 gRNA A2 DNA-targeting segment
  source 1..20: mol_type = other DNA
tatgagatcaacactcgcta

SEQ ID NO: 122 - DNA, 20 bp, synthetic construct
  misc_feature 1..20: note = Adamts5 gRNA B DNA-targeting segment
  source 1..20: mol_type = other DNA
ccaaggacttccccacgtta

SEQ ID NO: 123 - DNA, 20 bp, synthetic construct
  misc_feature 1..20: note = Adamts5 gRNA C DNA-targeting segment
  source 1..20: mol_type = other DNA
tgcttcccttatgcaagatt

SEQ ID NO: 124 - DNA, 20 bp, synthetic construct
  misc_feature 1..20: note = Adamts5 gRNA D DNA-targeting segment
  source 1..20: mol_type = other DNA
ttaggtaccctatttgaata

SEQ ID NO: 125 - DNA, 20 bp, synthetic construct
  misc_feature 1..20: note = Adamts5 gRNA E2 DNA-targeting segment
  source 1..20: mol_type = other DNA
tgcagtgggtgacaggtcca

SEQ ID NO: 126 - DNA, 20 bp, synthetic construct
  misc_feature 1..20: note = Adamts5 gRNA E DNA-targeting segment
  source 1..20: mol_type = other DNA
agggttatactgacgttgtg

SEQ ID NO: 127 - DNA, 20 bp, synthetic construct
  misc_feature 1..20: note = Adamts5 gRNA F DNA-targeting segment
  source 1..20: mol_type = other DNA
tgtctttcaaggagggctac

SEQ ID NO: 128 - DNA, 20 bp, synthetic construct
  misc_feature 1..20: note = Dpp4 gRNA A DNA-targeting segment
  source 1..20: mol_type = other DNA
actagtagacctgaggggtt

SEQ ID NO: 129 - DNA, 20 bp, synthetic construct
  misc_feature 1..20: note = Dpp4 gRNA B DNA-targeting segment
  source 1..20: mol_type = other DNA
gctccagtgtttaggccttg

SEQ ID NO: 130 - DNA, 20 bp, synthetic construct
  misc_feature 1..20: note = Dpp4 gRNA B2 DNA-targeting segment
  source 1..20: mol_type = other DNA
ggcaagctgaaaacgcatgc

SEQ ID NO: 131 - DNA, 20 bp, synthetic construct
  misc_feature 1..20: note = Dpp4 gRNA C DNA-targeting segment
  source 1..20: mol_type = other DNA
gtagatcgctttccactacc

SEQ ID NO: 132 - DNA, 20 bp, synthetic construct
  misc_feature 1..20: note = Dpp4 gRNA D DNA-targeting segment
  source 1..20: mol_type = other DNA
gaactccactgctcgtgagc

SEQ ID NO: 133 - DNA, 20 bp, synthetic construct
  misc_feature 1..20: note = Dpp4 gRNA E2 DNA-targeting segment
  source 1..20: mol_type = other DNA
ataggtgggcactattgaag

SEQ ID NO: 134 - DNA, 20 bp, synthetic construct
  misc_feature 1..20: note = Dpp4 gRNA E DNA-targeting segment
  source 1..20: mol_type = other DNA
atgggaaggtttataccagc

SEQ ID NO: 135 - DNA, 20 bp, synthetic construct
  misc_feature 1..20: note = Dpp4 gRNA F DNA-targeting segment
  source 1..20: mol_type = other DNA
cggtgtaaaaacaacgggaa

SEQ ID NO: 136 - DNA, 20 bp, synthetic construct
  misc_feature 1..20: note = Forward primer for SV 6.1 in Fig. 8
  source 1..20: mol_type = other DNA
ggaatgccaaggctactgtc

SEQ ID NO: 137 - DNA, 20 bp, synthetic construct
  misc_feature 1..20: note = Reverse primer for SV 6.1 in Fig. 8
  source 1..20: mol_type = other DNA
aaaagtctgctttgggtggt

SEQ ID NO: 138 - DNA, 21 bp, synthetic construct
  misc_feature 1..21: note = Forward primer for SV 6.3 in Fig. 8
  source 1..21: mol_type = other DNA
cttcatgaacctcactcagga

SEQ ID NO: 139 - DNA, 21 bp, synthetic construct
  misc_feature 1..21: note = Reverse primer for SV 6.3 in Fig. 8
  source 1..21: mol_type = other DNA
tctcggagtcaggatttacct

SEQ ID NO: 140 - DNA, 20 bp, synthetic construct
  misc_feature 1..20: note = Forward primer for SV 7.8 in Fig. 8
  source 1..20: mol_type = other DNA
tgtctctttgcctgttgctg

SEQ ID NO: 141 - DNA, 22 bp, synthetic construct
  misc_feature 1..22: note = Reverse primer for SV 7.8 in Fig. 8
  source 1..22: mol_type = other DNA
tctgctctacaaggcttacgtg

SEQ ID NO: 142 - DNA, 20 bp, synthetic construct
  misc_feature 1..20: note = Forward primer for SV 16 in Fig. 8
  source 1..20: mol_type = other DNA
caaccaggcagacttacagc

SEQ ID NO: 143 - DNA, 20 bp, synthetic construct
  misc_feature 1..20: note = Reverse primer for SV 16 in Fig. 8
  source 1..20: mol_type = other DNA
ggcctaggaaccagtcaaaa

SEQ ID NO: 144 - DNA, 23 bp, synthetic construct
  misc_feature 1..23: note = Forward primer for SV 25.5 in Fig. 8
  source 1..23: mol_type = other DNA
gcttactggaaagctacataggg

SEQ ID NO: 145 - DNA, 22 bp, synthetic construct
  misc_feature 1..22: note = Reverse primer for SV 25.5 in Fig. 8
  source 1..22: mol_type = other DNA
caacaacatagaaacccctgtc

SEQ ID NO: 146-147 - skipped (2 entries)

SEQ ID NO: 148 - DNA, 3155 bp, synthetic construct
  misc_feature 1..3155: note = Engineered Human Vk1-39Jk5 Locus
  source 1..3155: mol_type = other DNA
ggcgcgccgtagctttgaattttaaacatctatttgacaagaaatgcatagttccttctctttaaaataatgtaatgtttctttcaagaataagcttggtttgatgcctctctccccaacatgatagaagtgtagcataaatctatgaaaaattccatttccctgtgcctacaacaactacctgggattgaaaacttcttcccttgctctagtcctttcttctacacctacttccacatcatctgtgactcaaaacaatacttgtcaggaaagatcccggaaagagcaaaaaagacttccttagaggtgtcagagattcctatgccactatctgtcatctctagaaggggttgtgagtatgaggaagagcagagcttgtaaattttctacttgctttgacttccactgtatttcctaacaacaacaaccacagcaacacccataacatcacaggacaaacttctagtacttccaaggctttagtctcagtaaatcttctctacctccatcacagcagctagaaggtttgatactcatacaaatagtactgtagctttctgttcataattggaaaaatagacaagacccaatgtaatacaggctttccttcagccagttagcgttcagtttttggatcaccattgcacacatatacccagcatatgtctaatatatatgtagaaatccgtgaagcaagagttataatagcttgtgttttctattgtattgtattttcctcttatatcatcttcttcttcgttcattaaaaaaaaaccgttcaagtaggtctaaattaattattggatcataagtagataaaatattttatttcataacacattgacccgatgaatatgtttctttgccagacatagtcctcatttccaaggtaacaagcctgaaaaaattatactggagcaagtcaacaggtaatgatggtagcttttccttattgtcctggggcaagaataagacaaaagataacagggtagaataaagattgtgtaagaaagaaggacagcaacaggacatgggaaccttttatagagtaacattttgataatggatgatgagaattaatgagttagacagggatgggtgggaatgattgaaggtgtgagtactttagcacagattaagaccaaatcattaggatttaaagagttgtgtagagttagtgaaggaaaagccttagaattaaatttggctgcggataaaacattcttggattagactgaagactcttttctgtgctaagtaagtatatttatgataatgatgatgactgtagtgctgaatatttaataaataaaaacaaaattaattgccgcatacataatgtcctgaatactattgtaaatgttttatcttatttcctttaaactgtctacagcactataaggtaggtaccagtattgtcacagttacacagatatggaaaccgagacacagggaagttaagttacttgatcaatttcaagcaatcggcaagccatggagcatctatgtcagggctgccaggacatgtgactgtaaacagaagtttttcactttttaactcaaagagggtatgtggctgggttaatggaaagcttcaggaccctcagaaaacattactaacaagcaaatgaaaggtgtatctggaagattaagttttaacagactcttcatttccatcgatccaataatgcacttagggagatgactgggcatattgaggataggaagagagaagtgaaaacacagctttttatattgttcttaacaggcttgtgccaaacatcttctgggtggatttaggtgattgaggagaagaaagacacaggagcgaaattctctgagcacaagggaggagttctacactcagactgagccaacagacttttctggcctgacaaccagggcggcgcaggatgctcagtgcagagaggaagaagcaggtggtctttgcagctgaaagctcagctgatttgcatatggagtcattatacaacatcccagaattctttaagggcagctgccaggaagctaagaagcatcctctcttctagctctcagagatggagacagacacactcctgctatgggtgctgctgctctgggttccaggtgagggtacagataagtgttatgagcaacctctgtggccattatgatgctccatgcctctctgttcttgatcactataattagggcatttgtcactggttttaagtttccccagtcccctgaattttccattttctcagagtgatgtccaaaattattcttaaaaatttaaatgaaaaggtcctctgctgtgaaggcttttaaagatatataaaaataatctttgtgtttatcattccaggtgccagatgtgacatccagatgacccagtctccatcctccctgtctgcatctgtaggagacagagtcaccatcacttgccgggcaagtcagagcattagcagctatttaaattggtatcagcagaaaccagggaaagcccctaagctcctgatctatgctgcatccagtttgcaaagtggggtcccatcaaggttcagtggcagtggatctgggacagatttcactctcaccatcagcagtctgcaacctgaagattttgcaacttactactgtcaacagagttacagtacccctccgatcaccttcggccaagggacacgactggagattaaacgtaagtaatttttcactattgtcttctgaaatttgggtctgatggccagtattgacttttagaggcttaaataggagtttggtaaagattggtaaatgagggcatttaagatttgccatgggttgcaaaagttaaactcagcttcaaaaatggatttggagaaaaaaagattaaattgctctaaactgaatgacacaaagtaaaaaaaaaaagtgtaactaaaaaggaacccttgtatttctaaggagcaaaagtaaatttatttttgttcactcttgccaaatattgtattggttgttgctgattatgcatgatacagaaaagtggaaaaatacattttttagtctttctcccttttgtttgataaattattttgtcagacaacaataaaaatcaatagcacgccctaagatctagatgcatgctcgagtgccatttcattacctctttctccgcacccgacatagat

SEQ ID NO: 149 - DNA, 3166 bp, synthetic construct
  misc_feature 1..3166: note = Engineered Human Vk3-20Jk1 Locus
  source 1..3166: mol_type = other DNA
ggcgcgccgtagctttgaattttaaacatctatttgacaagaaatgcatagttccttctctttaaaataatgtaatgtttctttcaagaataagcttggtttgatgcctctctccccaacatgatagaagtgtagcataaatctatgaaaaattccatttccctgtgcctacaacaactacctgggattgaaaacttcttcccttgctctagtcctttcttctacacctacttccacatcatctgtgactcaaaacaatacttgtcaggaaagatcccggaaagagcaaaaaagacttccttagaggtgtcagagattcctatgccactatctgtcatctctagaaggggttgtgagtatgaggaagagcagagcttgtaaattttctacttgctttgacttccactgtatttcctaacaacaacaaccacagcaacacccataacatcacaggacaaacttctagtacttccaaggctttagtctcagtaaatcttctctacctccatcacagcagctagaaggtttgatactcatacaaatagtactgtagctttctgttcataattggaaaaatagacaagacccaatgtaatacaggctttccttcagccagttagcgttcagtttttggatcaccattgcacacatatacccagcatatgtctaatatatatgtagaaatccgtgaagcaagagttataatagcttgtgttttctattgtattgtattttcctcttatatcatcttcttcttcgttcattaaaaaaaaaccgttcaagtaggtctaaattaattattggatcataagtagataaaatattttatttcataacacattgacccgatgaatatgtttctttgccagacatagtcctcatttccaaggtaacaagcctgaaaaaattatactggagcaagtcaacaggtaatgatggtagcttttccttattgtcctggggcaagaataagacaaaagataacagggtagaataaagattgtgtaagaaagaaggacagcaacaggacatgggaaccttttatagagtaacattttgataatggatgatgagaattaatgagttagacagggatgggtgggaatgattgaaggtgtgagtactttagcacagattaagaccaaatcattaggatttaaagagttgtgtagagttagtgaaggaaaagccttagaattaaatttggctgcggataaaacattcttggattagactgaagactcttttctgtgctaagtaagtatatttatgataatgatgatgactgtagtgctgaatatttaataaataaaaacaaaattaattgccgcatacataatgtcctgaatactattgtaaatgttttatcttatttcctttaaactgtctacagcactataaggtaggtaccagtattgtcacagttacacagatatggaaaccgagacacagggaagttaagttacttgatcaatttcaagcaatcggcaagccatggagcatctatgtcagggctgccaggacatgtgactgtaaacagaagtttttcactttttaactcaaagagggtatgtggctgggttaatggaaagcttcaggaccctcagaaaacattactaacaagcaaatgaaaggtgtatctggaagattaagttttaacagactcttcatttccatcgatccaataatgcacttagggagatgactgggcatattgaggataggaagagagaagtgaaaacacagctttttatattgttcttaacaggcttgtgccaaacatcttctgggtggatttaggtgattgaggagaagaaagacacaggagcgaaattctctgagcacaagggaggagttctacactcagactgagccaacagacttttctggcctgacaaccagggcggcgcaggatgctcagtgcagagaggaagaagcaggtggtctttgcagctgaaagctcagctgatttgcatatggagtcattatacaacatcccagaattctttaagggcagctgccaggaagctaagaagcatcctctcttctagctctcagagatggagacagacacactcctgctatgggtgctgctgctctgggttccaggtgagggtacagataagtgttatgagcaacctctgtggccattatgatgctccatgcctctctgttcttgatcactataattagggcatttgtcactggttttaagtttccccagtcccctgaattttccattttctcagagtgatgtccaaaattattcttaaaaatttaaatgaaaaggtcctctgctgtgaaggcttttaaagatatataaaaataatctttgtgtttatcattccaggtgccagatgtataccaccggagaaattgtgttgacgcagtctccaggcaccctgtctttgtctccaggggaaagagccaccctctcctgcagggccagtcagagtgttagcagcagctacttagcctggtaccagcagaaacctggccaggctcccaggctcctcatctatggtgcatccagcagggccactggcatcccagacaggttcagtggcagtgggtctgggacagacttcactctcaccatcagcagactggagcctgaagattttgcagtgtattactgtcagcagtatggtagctcaccttggacgttcggccaagggaccaaggtggaaatcaaacgtaagtaatttttcactattgtcttctgaaatttgggtctgatggccagtattgacttttagaggcttaaataggagtttggtaaagattggtaaatgagggcatttaagatttgccatgggttgcaaaagttaaactcagcttcaaaaatggatttggagaaaaaaagattaaattgctctaaactgaatgacacaaagtaaaaaaaaaaagtgtaactaaaaaggaacccttgtatttctaaggagcaaaagtaaatttatttttgttcactcttgccaaatattgtattggttgttgctgattatgcatgatacagaaaagtggaaaaatacattttttagtctttctcccttttgtttgataaattattttgtcagacaacaataaaaatcaatagcacgccctaagatctagatgcatgctcgagtgccatttcattacctctttctccgcacccgacatagat

SEQ ID NO: 150 - DNA, 82 bp, synthetic construct
  misc_feature 1..82: note = Guide RNA Scaffold v1
  source 1..82: mol_type = other DNA
gttggaaccattcaaaacagcatagcaagttaaaataaggctagtccgttatcaacttgaaaaagtggcaccgagtcggtgc

SEQ ID NO: 151 - DNA, 76 bp, synthetic construct
  misc_feature 1..76: note = Guide RNA Scaffold v2
  source 1..76: mol_type = other DNA
gttttagagctagaaatagcaagttaaaataaggctagtccgttatcaacttgaaaaagtggcaccgagtcggtgc

SEQ ID NO: 152 - DNA, 86 bp, synthetic construct
  misc_feature 1..86: note = Guide RNA Scaffold v3
  source 1..86: mol_type = other DNA
gtttaagagctatgctggaaacagcatagcaagtttaaataaggctagtccgttatcaacttgaaaaagtggcaccgagtcggtgc